European Patent Application EP 4 335 452 A1, published March 13, 2024. Title: Pharmaceutical Composition for enhancing anticancer effects of anticancer drugs. Applicant: L-Base Co., Ltd. The sequence listing filed with the application follows.

SEQUENCE LISTING (1 sequence)

SEQ ID NO: 1 - protein, 8 aa, Artificial Sequence
  Oligopeptide AQTGTGKT
AQTGTGKT